European Patent Specification EP 3 604 502 B1, published January 1, 2025. Title: Stable production of highly virulent enterovirus 71 and use thereof. Applicant: Tokyo Metropolitan Institute of Medical Science. The sequence listing filed with the application follows.

SEQUENCE LISTING (21 sequences)

SEQ ID NO: 1 - DNA, 18 bp, Artificial Sequence
  EXT1-sgRNA sense
caccacccacaacacatc

SEQ ID NO: 2 - DNA, 17 bp, Artificial Sequence
  EXT1-sgRNA antisense
aaaccatttcctccttc

SEQ ID NO: 3 - DNA, 22 bp, Artificial Sequence
  EXT2-sgRNA sense
cacccttcaattcaccaatcca

SEQ ID NO: 4 - DNA, 18 bp, Artificial Sequence
  EXT2-sgRNA antisense
aaacctatttacattaac

SEQ ID NO: 5 - DNA, 48 bp, Artificial Sequence
  EV71 Isehara 5'-primer
cggcggccgcgtaatacgactcactataggttaaaacagcctgggttg

SEQ ID NO: 6 - DNA, 39 bp, Artificial Sequence
  EV71 Isehara 3'-primer
tactcactttttttttttttttttttttttttctattct

SEQ ID NO: 7 - DNA, 7434 bp, Enterovirus 71 Isehara strain
ttaaaacagcctgtgggttgcacccacccacagggcccactgggcgccagcactctggtactgaggtacctttgtgcgcctgtttttacttcccctccccgaagtaacttagaagctgtaaatcaacgatcaatagtaggtgtgacacaccagtcacactttggtcaagcacttctgtttccccggactgagtatcaataggctgctcgcgcggctgaaggagaaaacgttcgttacccgaccaactacttcgagaagcttagtaccaccatgaacgaggcagagtgtttcgttcagcacaaccccagtgtagatcaggctgatgagtcactgcaacccccatgggcgaccatggcagtggctgcgttggcggcctgcccatggagaaatccatgggacgctctaattctgacatggtgcgaagagcctattgagctagttggtagtcctccggcccctgaatgcggctaatcctaactgcggagcacatgctcacaaaccagtgggtggtgtgtcgtaacgggcaactctgcagcggaaccgactactttgggtgtccgtgtttccttttattcttatattggctgcttatggtgacaatcaaagaattgttaccatatagctattggattggccatccagtgtgcaacagagcaattgtttatctattcattggtttcgtacctttatcactgaagtctgtgatcactcttaaattcattttgaccctcaatacaattaaacatgggctcacaggtgtccacacagcgctccggttcgcatgaaaattctaactcagccaccgagggttccaccataaattatactaccattaattactataaagactcctatgccgccacagcaggtaaacagagccttaagcaggacccagacaagtttgcaaatcctgtcaaagacatcttcactgaaatggcagcgccattaaaatctccatctgctgaggcatgtggttacagcgatcgggtagcacagttaactattggcaactctaccatcactacgcaagaagcagcaaacatgatagttggctatggtgagtggccatcctactgctcggattctgacgccacagcagtggacaaaccaacgcgcccagatgtttcagtgaataggttttatacattggacactaaattgtgggagaaatcatccaaggggtggtactggaaattcccggatgtgttgactgaaaccggggtcttcggtcaaaatgcacaattccactacctctatcggtcgggattctgcattcacgtgcagtgcaatgctagtaagttccaccaaggagcactcctagtcgctgtcctcccagaatatgtcattgggacagtagcaggtggcacagggacggaggatagtcaccccccttacaagcagactcaacccggtgctgatggctttgaattgcaacacccgtacgtgcttgatgctggcattccaatatcacaattaacagtgtgcccacaccagtggattaatttgaggactaacaattgtgccacaataatagtaccgtacataaacgcactaccctttgattctgccttgaaccattgcaactttggtctgctggttgtgcctattagcccgttagattatgaccaaggtgcgacgccagtgatccccattactatcacattggccccaatgtgctctgaatttgcaggccttaggcaagcagttacgcaagggtttcctactgagctgaaacccggcacaaaccaatttttaaccactgacgatggcgtctcagcacccattctgccaaactttcaccccaccccgtgtatccatatacccggtgaagttagaaacttgctagagctatgccaggtggagaccatcttagaggttaacaatgtacccacgaatgccactagcttaatggagaggctgcgcttcccggtctcagcccaagccgggaaaggtgaactatgtgcagtgttcagagctgaccctgggcgaaatggaccatggcagtccaccctgttgggtcagttgtgtgggtattacacccaatggtcaggatcactggaagtcaccttcatgtttactgggtcctttatggctactggcaagatgctcatagcatacacaccaccaggaggccccttacccaaggaccgggcgaccgccatgttgggtacacacgtcatctgggactttgggttgcaatcgtctgtcacccttgtaataccatggatcagcaacactcactacagagcgcacgctcgagatggtgtgttcgattactacactacaggtttggttagcatatggtaccagacgaattacgtggttccaattggggcacctaatacagcctacataatagcattggcggcagcccagaagaatttcaccatgaagttgtgtaaggatgctagtgatatcctacagacaggcactatccagggagacagggtggcagatgtgattgagagttctataggggatagtgtgagcagagccctcacccaagctttaccggcacctacaggccaaaacacgcaggtaagcagccaccgattagacactggtaaagttccagcactccaagccgctgaaattggagcatcatcaaatgccagcgatgagagtatgattgagacacgatgtgttcttaattcacacagcacagctgagaccactcttgatagcttcttcagtagagcgggattagttggagagatagacctccctcttgaaggcacaaccaacccgaatgggtatgcaaattgggacatagacataacaggttacgcgcaaatgcgtagaaaggtggagctgtttacctacatgcgttttgacgcagagttcaccttcgtagcgtgcacgcctaccggggaagttgtcccgcaattgctccaatatatgtttgtaccacctggagcccccaagccagactctagagaatctcttgcatggcaaactgccactaatccctcagtctttgtgaagctgtcagaccccccagcacaggtttcagttccattcatgtcacctgcaagcgcctaccaatggttttatgacgggtatcccacattcggtgaacacaagcaggaaaaagaccttgaatatggggcatgcccaaacaacatgatgggtacgttctcggtgcggactgtaggaacctcgaagtccaagtacccattggtgatcaggatttacatgaggatgaagcacgtcagggcgtggatacctcgcccaatgcgtaaccaaaactacttatttaaagccaacccaaattatgctggtaactccattaaaccaactggtaccagtcgcacagcgatcaccactctcgggaaatttggacagcaatccggggctatctacgtgggcaactttagagtggttaaccgccaccttgctactcataatgactgggcaaaccttgtttgggaagacagctcccgcgacttgctcgtatcatctacctctgcccaaggttgtgacacgattgctcgttgcaactgtcagacaggagtgtattactgtaactcaatgagaaaacactatccggtcagtttctcgaagcccagtttgatcttcgtagaggccagcgagtattaccctgctagataccagtcacaccttatgcttgcagtgggtcactcggagccaggggattgcggtggcattcttagatgccaacacggtgtcgtagggatagtttccaccgggggaaacggcctagtggggttcgccgatgtgagggatcttctgtggttggatgatgaggccatggagcagggcgtgactgattacattaaagggcttggagatgcttttggcatggggtttacagacgcagtgtcaagagaagttgaagcattgaaaaatcacttgatcggctcagagggtgccgtggagaggatccttaagaacttagttaaactcatctctgcgctcgtcattgtcatcaggagtgattatgacatggtcacattgacggcaacacttgccctgatcgggtgtcacggcagcccttgggcctggattaagtcgaaaacagcgtcgattttgggcataccgatggctcaaaagcagagtgcctcttggttaaagaagttcaacgatgcggcgagtgccgccaaggggcttgagtggatctccaacaaaatcagcaaatttatcgattggctcaaggagaaaattatcccggctgctaaagagaaagtcgagtttctaaacaatctaaagcaactccccttattggagaaccaaatttctaatctcgaacagtcagcagcttcccaggaggacctcgaagcgatgtttggcaacgtgtcttatctggcccacttctgccgcaaattccaacccctctatgccacggaagcaaagagggtgtatgccctagaaaagagaatgaataattacatgcagttcaagagcaaacaccgtattgaacctgtatgcctgattatcagaggctcgcctggcactgggaagtccttggcaacagggattattgctagagctatagctgacaagtaccactccagtgtgtattccttacctccggacccagatcactttgatggatacaagcaacagatcgttactgttatggatgatctatgccaaaacccggacgggaaagacatgtcactattttgtcagatggtctccacagtggattttataccgcctatggcatctctggaggagaagggagtctcattcacctccaagtttgtgattgcctccactaacgccagtaacatcatagtgccaacagtctcggattcagatgccatccgtcgtcggttcttcatggactgcgatattgaggtgaccgattcctataagacagagctgggtaggcttgatgcagggagagcagctaggctgtgctctgagaacaacactgcaaactttaaacggtgcagcccattagtctgtgggaaagcaatccagcttagggataggaagtctaaggtgagatacagtgtggacacggtggtgagtgagcttatcagggagtataacaacagatcagctattgggaataccatcgaagctcttttccaaggaccccctaaatttagaccgataaggattagcctagaggagaagcccgcacctgatgctattagtgacctattagctagtgtcgatagtgaagaggttcgccaatactgtagagatcagggatggattgtacctgattctcccaccaacgttgagcgccacttgaatagagctgtcttgatcatgcaatctatagccaccgtggtagcggttgtgtcccttgtttatgtcatctacaagttgttcgccggttttcaaggagcatattccggcgcccctaagcaagcactcaagaaaccagtgttgcgtacggcaactgtgcaggggccaagcttggacttcgccctatctctacttaggaggaacatcaggcaggtccaaaccgaccagggccactttacaatgttaggagtgcgagaccacttggctgtgctccccagacactcccaaccaggaaagaccatctgggttgaacacaaattagtgaagatcgtggatgctgtggagctagtagatgagcaaggagttaacctagagctcacactggtgacgcttgacaccaacgaaaaatttagagacatcacaagattcataccagaaacaattagtcctgctagtgatgccactttagttataaatactgaacatatgcccaatatgtttgtgccagttggagatgtagtccagtatggatttttgaaccttagtggtaagcccactcacaggactatgatgtacaatttcccaacaaaagcaggacagtgtggtggtgtcgtgactgctgtgggtaaagtgattgggatccacattggtggcaacggtaggcagggtttctgcgctgccctgaagagaggatacttttgcagcgaacaaggtgagatccaatggatgaagcccaacaaagaaactggcaggttaaacatcaacggacctactcgcactaaacttgaaccaagtgtctttcatgatgtgttcgagggcactaaagagccagcagtgctgactagtaaagacccaaggctggaggttgactttgaacaggctcttttttcaaaatacgtgggaaacacgcttcatgaacctgacgagtttgtcaaggaggcggccttacattatgccaaccaactcaagcagttagatattaagaccaccaagatgagcatggaggatgcttgttacggtacagagaacctggaagctatagaccttcacacaagtgcaggatatccatacagtgcactgggcatcaagaaaagggatattttggacccaacaactcgcgatgtcagcaagatgaaattttacatggacaagtatgggttagatctaccgtactccacttatgttaaagatgaactcagggccatcgacaaggtcaagaaagggaagtctcgtctcatagaagcgagcagtctaaatgactcagtgtacttgagaatgacatttgggcacctttatgaaacttttcatgccaatccaggtacagtcactggttcagctgttggatgcaatccagatgtgttctggagtaagttgccaattctacttccaggatcgctttttgcatttgactactcggggtatgacgctagtctcagcccagtgtggttcagggcgctggagatagtcctacgggaaattgggtactccgaggacgcagtgtctctcatagaagggatcaatcacactcaccatgtgtaccgcaataaaacttattgtgttcttgggggaatgccctcaggttgctcaggcacctccattttcaactcgatgatcaataacatcattattaggacactcctgattaaaacattcaaagggatagatctagatgaattgaatatggtggcctacggggatgatgtgttggctagttaccccttcccaattgactgtctggaattggcaagaacaggcaaggagtatggtttaactatgacccctgccgacaagtcaccttgctttaatgaagttacatgggagaatgccactttcttgaagagaggattcttgcctgatcatcaattcccgttcctcatccaccccacgatgccaatgagggagattcacgaatctattcgttggactaaagatgcacgaagtactcaagatcacgtgcgctctctctgcttattagcatggcacaacgggaaagaggagtatgaaaaatttgtgagtacaatcagatcagttccaattggaaaggcattggctataccgaattttgagaatctgagaagaaattggctcgaattgttttaaatttacagtttgtaactgaaccctaccagtaatctggtcgtgttaatgactggtgggggtaaatttgttataaccagaatagcaaaaaaaaaaaaaaaaaaaaaaaaa

SEQ ID NO: 8 - DNA, 15 bp, Artificial Sequence
  Sequencing primer (F)
  misc_feature (2)..(2): n is a, c, g, or t
cnayayaatatatta

SEQ ID NO: 9 - DNA, 18 bp, Artificial Sequence
  Sequencing primer (R)
  misc_feature (2)..(2): n is a, c, g, or t
  misc_feature (5)..(5): n is a, c, g, or t
  misc_feature (11)..(11): n is a, c, g, or t
anacnarrttncccatca

SEQ ID NO: 10 - DNA, 7430 bp, Enterovirus 71 Y90-3896 strain
ttaaaacagcctgtgggttgcacccacccacagggcccactgggcgccagcactctggtacttaggtacctttgtgcgcctgttttatctcccttcccccgaagtaacttagaagctgtgagctaacgatcaacagtaggtgtgacataccagtcatatcttgatcaagcacttctgtttccccggactgagtatcaataggctgctcgcgcggctgaaagagaaaacgttcgtcacccggccaactacttcgagaagcttagtaccaccatgaacgaggcagagtgtttcgctcggcacaaccccagtgtagatcaggctgatgagtcactgcaatccccatgggcgaccatggcagtggctgcgttggcggcctgcccatggagaaatccatgggacgctctaattctgacatggtgcgaagagcctattgagctagctggtagtcctccggcccctgaatgcggctaatcctaactgcggagcacacacccacaagccagtgggcagtgtgtcgtaacgggcaactctgcagcggaaccgactactttgggtgtccgtgtttccttttattcttgtattggctgcttatggtgacaatcaaagagttgttaccatatagctattggattggccatccggtgtgcaacagagcaattatttacctatttattggttttgtaccattgacactgaagtctgtgattacccttaattttattttgaccctcaacacagtcaaacatgggctcacaggtgtccacacaacgctccggctcacatgaaaactctaactcagctactgagggctccaccataaactacactactattaattactacaaggactcctatgccgctacagcaggcaaacagagcctcaagcaggatccagataagtttgcaaatcctgtcaaagatattttcactgaaatggcagcgccactaaagtccccatccgctgaagcatgtggatacagcgaccgagtagcgcagttaactattggcaactctaccatcactacacaagaagcagcaaacattatagttggctatggtgaatggccctcctactgctcggattctgacgctacagcagtggacaaaccaacgcgcccagatgtttcggtgaacaggttttacacattggacaccaaattatgggagaaatcgtccaagggatggtactggaaattcccggatgtgttaacagaaaccggggtttttggccagaatgcacaattccattacctctatcggtcagggttctgcattcacgtgcaatgcaatgctagcaaattccatcagggagcgctcctagtcgctgttctcccggagtatgtcattgggacagtggcgggtggcacagggacggaggatagccaccccccttacaagcagactcaacccggcgctgatggttttgagttacaacatccgtacgtgcttgacgctggcattccaatatcacaattaacagtgtgcccacatcagtggattaacttgaggaccaacaattgtgccacaataatagtgccatacattaatgcactgccctttgattctgccttaaaccattgtaactttggcctactggttgtgcccattagcccgttggacttcgaccaaggagcgacgccagtgatccccattactatcacattggccccaatgtgttctgaatttgcaggtcttaggcaagcggtcacgcaaggatttcctactgagctgaaacctggcacaaaccaatttttaaccactgacgatggcgtttcagcgcccattctgccaaactttcaccccaccccatgcatccatatacctggtgaggttagaaatttgctagagctatgccaggtggagactatcttagaggtcaacaatgtacccacgaatgccactagtttaatggagagactgcgctttccggtctcagcccaagcaggaaaaggcgagttgtgtgcagtgttcagagccgatcctgggcgaaatgggccttggcaatctaccttgttgggccagttgtgcgggtactacactcaatggtcaggatcactggaagtcacgttcatgttcactgggtcctttatggccaccggcaagatgcttatagcttacacgccaccaggaggccctttgcccaaggaccgggcgaccgccatgttgggtacgcatgtcatctgggattttgggctgcaatcgtctgtcacccttgtaataccatggatcagcaacactcattacagagcgcatgctcgagatggggtgttcgactattacactacaggcctggttagtatatggtatcagacgaactatgtggttcccattggagcacccaatacagcctatataatagcgttagcggcagcccagaagaattttaccatgaaattgtgtaaggatgccagtgatatcttacagacaggcactattcagggggatagggtggcagatgtgattgagagttctataggggatagtgtgagcagagctctcactcaagctctaccggcacccacaggccaggacacgcaggtaagcagccatcgattggatactggcaaagttccagcactccaagccgctgagattggagcatcatcaaatgctagtgatgagagtatgattgagacacgatgtgttcttaattcgcacagcacagctgagaccactctcgatagtttcttcagcagagcgggattagttggggagatagaccttcctcttgaaggcacaaccaacccaaatggttatgcaaattgggacatagatataacaggttatgcgcagatgcgtagaaaggtggagctgttcacctacatgcgttttgacgcagaattcaccttcgtcgcgtgcacgcccaccggggaggttgtcccacaattactccaatatatgtttgtgccacctggggcccccaagccagaatccagagaatccctcgcatggcaaactgccaccaatccctcggtttttgttaagctatcagaccccccagcgcaggtttcagttccattcatgtcacctgcgagtgcttaccaatggttttatgacggatatcccacgttcggtgaacacaagcaggaaaaagaccttgaatacggggcatgtccaaacaacatgatgggcacgttctcagtgcggaccgtaggaacctcgaagtccaagtaccctttagtaattaggatttatatgaggatgaagcacgtcagggcatgggtacctcgtccaatgcgcaaccaaaactatctattcaaagccaacccaaattacgccggcaactccattaagccaaccggtgccagtcgcacagcgatcaccactctcggaaaatttgggcaacaatccggggccatctatgtgggtaactttagagtggttaatcgccatcttgccactcacaatgattgggcgaaccttgtttgggaagacagctctcgcgacttactcgtatcatctaccaccgctcagggttgtgatacgatagcccgttgcgattgtcagacaggagtgtactattgtaactcaaggagaaaacactacccggttagtttctcaaaacccagcttgatctttgtagaggccagcgagtactacccagccaggtatcagtcacacctcatgctcgcagtgggtcactcagaaccaggagattgcggtggcatactcagatgccaacacggtgttgtagggatagtttctaccgggggaaatggcctggtggggttcgccgacgtgagggaccttctgtggttggatgatgaagccatggaacagggtgtgtctgattacattaaagggcttggtgatgctttcggcatgggattcacagacgcagtgtcaagagaggttgaagccttgaaaagtcatttgatcggttcagagggcgccgtggagaagattcttaagaacttagtaaaactcatctctgcgcttgtcattgtcatcaggagtgactacgacatggtcacattgacggcaacgcttgccctgattgggtgccatgggagcccttgggcctggattaagtcgaaaacagcttcaattttgggtataccaatggcccagaagcagagcgcctcttggttaaagaagttcaacgatgcggcgagtgccgctaaggggcttgagtggatctccaataaaatcagtaaatttatcgattggctcaaggagaaaatcatcccggctgctaaagaaaaagtcgaatttctaaataacttgaagcaacttcctttattggaaaaccaaatctctaaccttgaacagtcagcagcttcgcaggaggaccttgaagcgatgtttggcaacgtgtcctacttggcccacttttgccgcaaattccaacctctctatgccacagaagcaaagagggtgtacgccttagaaaaaagaatgaacaattacatgcagttcaagagcaaacaccgtattgaacctgtgtgcttgatcattagaggctcacctggtactgggaagtctttagcaacagggattatcgctagagctatagcagataagtatcactctagtgtgtattccctacctccagacccagatcattttgatggatataaacaacagattgtcactgttatggatgacctctgccaaaatccggatgggaaagacatgtcactattctgtcagatggtttccacagtggactttataccgcctatggcatccctggaggagaagggagtctcattcacctccaagtttgtgattgcctccactaacgctagcaacatcatagtaccaacagtctcggattcagatgccatccgtcgtcggttctttatggactgtgatattgaagtgaccgattcctataagacagatttgggtaggcttgatgcagggagagcggccaggctgtgttctgagaacaacactgcaaatttcaaacggtgcagcccactagtatgtgggaaagcaatccagcttagggatagaaagtccaaggtgagatacagtgtggacacagtggtgagtgagctcattagggaatataacaacaggtcagctattgggaataccatcgaagctctttttcaggggccccctaaattcagaccgataaggattagtctggaggagaagcccgcacctgacgctatcagtgatctgctggctagtgttgatagtgaagaagtccgccaatactgtagagatcaaggatggattgtgcctgatactcccaccaacgttgagcgccacttgaatagagctgtcttgattatgcaatctgtagccaccgtggtggcagttgtgtcccttgtttacgtcatctacaagttgtttgccggtttccaaggagcatattccggcgcccccaagcaaacacttaagaaaccggtgctgcgtacagcaaccgtgcagggaccgagcttggacttcgccctatctttactcagaaggaacattaggcaggtccaaaccgatcagggccacttcacaatgctaggagtgcgggaccacttggctgtactccctagacactcccaaccaggaaagaccatttgggttgagcacaaactggtgaagatcgtagacgccgtggagttggtagatgaacaaggggttaacctagagcttacactggtaacgcttgacaccaatgaaaaattcagagacatcacaaggttcataccagaaacaattagtcctgctagtgatgccactctagtcataaatactgaacatatgcccagcatgtttgtgccggttggagatgtggtccagtatggatttttgaatcttagtggcaagcccactcaccggactatgatgtacaacttcccaacaaaggcaggacagtgtggtggtgttgtgactgctataggtaaagtgattgggatccacattggtggtaatggtaggcaaggtttctgtgctgctctgaagagggggtacttttgtagtgaacagggtgagatccagtggatgaagcccaacaaagaaactggcaggttgaacatcaatgggcctactcgcaccaagcttgagccaagtgttttccatgatgtgttcgagggcaccaaagagccagcagtgctgactagcaaagacccaaggctggaagtcgactttgagcaggctttgttctcaaaatatgtaggaaacacgcttcacgagcccgacgagtttgtcagggaggcggctttgcactatgccaaccaactcaaacagttagatatcaaaaccaccaaaatgagcatggaggatgcttgttatggtacagagaacctggaagctatagatcttcacactagtgcgggatacccatacagtgcactaggcattaagaaaagggatattttggatccaataactcgtgatgttagtaaaatgaaattctacatggacaaatatgggttggatctaccgtattccacttatgtcaaagatgaactcagggccattgataagatcaagaaagggaagtcccgtctcatagaagcgagcagtctaaatgactcagtgtacttaaggatgacatttgggcacctttatgaaaccttccacgccaatccgggtacagtcactggttcagctgttggatgcaacccagatgtgttttggagtaagttaccaattctactcccaggatcgctttttgcgtttgactactcggggtatgacgccagtctcagcccagtgtggtttagggcgttggagatagtcctgcgggaaattggatactctgaggacgcagtgtctctcatagaagggatcaatcacacccaccatgtgtatcgcaataaaacttattgtgttcttgggggaatgccctcaggttgctcaggcacttccattttcaactcgatgatcaataatatcattatcaggacactattgattaaaacattcaaagggatagatctagatgaattgaatatggtggcctacggggatgatgtgttagctagttatcccttcccaattgactgtctagagctggcaaagacaggcaaggagtatggcttgactatgacccctgccgacaaatcaccctgctttaatgaagttacgtgggagaatgccaccttcttaaagagaggatttctgcctgatcatcaatttccgttcctcatccaccctacgatgccaatgaaggaaattcacgagtccattcgctggaccaaagacgcacgaaatacccaagatcacgtgcgctccctctgcttgttagcatggcacaacgggaaagaggagtatgaaaaatttgtgagcgcaatcagatcggttccaattgggaaagcgttagccctaccaaattttgagaatctgaggagaaattggctcgaattgttttaaatttacagtttgtaactgaaccccaccagaaatctggtcgcgttaatgactggtgggggtaaatttgttataaccagaatagcaaaaaaaaaaaaaaaaaaaaa

SEQ ID NO: 11 - DNA, 7433 bp, Enterovirus 71 N772 strain
ttaaaacagcctgtgggttgtacccactcacagggcccactgggcgctagcactctggtatctcggtacctttgtgcgcctgttttataccccccccccctcagtgaaacttagaagcagcaaacaacgatcaatagcagacataacactccagttatgtctcgatcaagcacttctgtttccccggaccgagtatcaatagactgctcgcgcggttgaaggagaaaacgttcgttatccggctaactacttcgggaaacctagtaacaccatgaaagttgcggagagcttcgttcagcactcccccagtgtagatcaggtcgatgagtcaccgcattccccacgggcgaccgtggcggtggctgcgttggcggcctgcccatggggtaacccatggggcgctctaatacggacatggtgcgaagagtctactgagctagttagtagtcctccggcccctgaatgcggctaatcccaactgcggagcacacgcccacaagccagcgggtagtgtgtcgtaacgggcaactctgcagcggaaccgactactttgggtgtccgtgtttccttttatctttatattggctgcttatggtgacaattaaagaattgttaccatatagctattggattggccatccggtgtgcaacagagcaattgtttacctatttattggttttgtaccattgaccttgaagtctgtgattacccttagttatatcttgaccctcaacacagctaaacatgggttcgcaggtgtctacacagcgctccggttctcacgaaaactcaaactcagccactgaaggttccaccataaactacaccaccattaattactacaaagactcctatgctgccacagcaggcaaacagagtctcaagcaggatccagacaagtttgcaaatcctgttaaagacatcttcactgaaatggcagcgccactgaaatctccatccgctgaggcatgtggatacagcgatcgagtggcgcaattaaccattggcaactccaccatcaccacgcaagaagcggctaacatcatagttggttatggtgagtggccttcctactgctcggattctgacgctacagcagtggataaaccaacgcgcccggatgtttcagtgaacaggttttatacattggacaccaagttgtgggagaaatcgtccaagggatggtactggaagttcccggatgtgttaactgaaaccggggtttttgggcaaaatgcacaattccactacctctaccgatcagggttctgtattcacgtgcagtgcaatgctagtaaatttcaccaaggagcactcctagttgctgtcctaccagagtacgtcattgggacagtggctggcggtacagggacggaagacagtcaccctccttacaagcagactcaacccggcgccgatggcttcgaattgcaacacccgtacgtgcttgatgctggcatcccaatatcacagttaacagtgtgcccacaccagtggattaatttgaggaccaacaattgtgctacaataatagtgccatacattaacgcactaccttttgattctgctttgaaccactgtaactttggcctattagttgtgcctattagcccgctagattacgaccaaggagcgacgccagtaatccctataactatcacattggccccaatgtgttctgaattcgcaggtctcaggcaagcagtcacgcaagggtttcccaccgagctgaaacctggcacaaatcaatttttaaccactgatgatggcgtttcggcacctattctaccaaacttccaccccaccccctgtatccacatacctggtgaagttaggaacttgctagagttatgccaggtggagaccattttggaggtcaacaatgtgcccacgaatgccactagcttaatggagaggctgcgctttccggtctcagcacaagcagggaaaggcgagctgtgtgcggtgttcagagccgatcctgggcgaaatggaccgtggcagtccaccttgctgggtcagttgtgcgggtattatacccaatggtcaggatcattggaggtcaccttcatgttcactggatccttcatggctactggcaagatgctcatagcctatacaccgccgggaggccctttgcccaaggaccgggcaaccgccatgttgggcacgcacgtcatctgggattttgggctgcaatcgtctgttacccttgtgataccatggatcagcaacactcactacagagcgcatgcccgagatggagtgtttgactactacaccacagggttagtcagtatatggtatcagacaaattacgtggttccaattggggcgcccaatacagcctatataatagcattagcggcagcccaaaagaacttcactatgaaattgtgcaaggatgctagtgatatcctgcagacgggcaccatccagggagatagggtggcagatgtaattgagagttccataggggatagtgtgagcagagccctcactcaagctctaccagctcccacaggccagaacacacaggtgagcagtcatcgactggatacaggtaaggttccagcactccaagctgctgagattggagcatcatcaaatgctagtgatgagaacatgattgagacacgctgtgttcttaactcgcacagcacagctgagaccactcttgatagtttcttcagcagagcgggattagttggagagatagatctcccccttgaaggcacaaccaacccaaatggctatgccaactgggacatagatataacaggttacgcgcaaatgcgtagaaaggtggagctattcacctacatgcgctttgatgcagagttcacttttgttgcgtgcacacccaccggggaagttgtcccacaattgctccaatatatgtttgtgccacctggagcccctaagccagattccagggaatcccttgcatggcaaactgccaccaacccctcagtttttgtcaagctgtcagaccctccagcgcaggtttcagtaccattcatgtcacctgcgagtgcttaccaatggttttatgacggatatcccacatttggagaacataaacaggagaaagatcttgaatatggggcatgtcctaacaacatgatgggcacgttctcagtgcggactgtagggacttccaagtccaaataccctttagtggttaggatttacatgagaatgaagcacgtcagggcgtggatacctcgcccgatgcgcaaccaaaactacctattcaaagccaacccaaattatgctggcaactccattaagccaactggtaccagtcgcacggcgatcactactcttgggaaatttgggcaacagtctggggccatttacgtgggtaactttagagtggttaaccgtcatcttgccactcataatgattgggcaaatcttgtttgggaagacagctctcgcgacttgctcgtgtcatccaccactgcccaaggttgtgacacgattgcccgttgcaattgccagacaggggtgtactattgtaattcaagaagaaaacactacccagtcagtttttcaaaacccagcctgatctatgtagaggctagcgagtattacccagccaggtaccagtcacatctcatgctcgcacagggccactcagaacctggtgattgtggtggtatccttagatgccaacatggtgtcgtcggtatagtgtctactggtggcaatgggctcgttggctttgcagacgtcagggacctcttgtggttagatgaagaagctatggagcagggcgtgtccgactacatcaagggtctcggagatgctttcgggacaggtttcactgatgcagtctcaagggaggttgaagctctcaagaactatcttatagggtctgaaggagcagttgaaaaaattctaaaaaatcttattaaactaatctctgcactggtgattgtaatcagaagtgattacgacatggttacccttactgcaaccctagcgctgataggttgtcatggcagtccttgggcttggatcaaagccaaaacagcttctatcttaggcatccctatcgctcagaagcaaagcgcttcttggctcaagaaattcaatgacatggccaacgctgctaaggggttagagtgggtttctaataagatcagcaaattcattgattggcttaaggagaaaatagtaccagcagctaaggagaaggttgaattcctaaataacttgaaacagttgccattgctagagaatcagatctcaaacttggaacaatctgctgcctcacaagaggaccttgaagtcatgtttgggaatgtgtcgtatctagcccacttctgtcgcaagttccagccgctatacgccacggaagctaaaagggtttatgccctggagaagagaatgaataactatatgcagttcaagagcaaacaccgaattgaacctgtatgtcttattattaggggctcaccaggcactgggaagtctttagccactggtatcattgctcgagcaatcgctgacaagtaccactccagcgtgtactcgcttccaccagacccagatcattttgatggctacaagcaacaggtggttacagtgatggatgacttgtgtcaaaaccccgatggcaaggatatgtccttattctgtcaaatggtatccaccgtagacttcatcccaccaatggcttctcttgaggagaagggagtttccttcacctctaagtttgttatcgcatctactaatgccagtaacatcatagtgccaacagtgtctgactctgacgctattcgccgcaggttctacatggattgtgatattgaagtgacagactcgtacaaaactgatctaggtagactggatgcagggcgagccgccaaactgtgctctgagaacaacactgcaaatttcaaacgttgcagcccattagtgtgtgggaaagctatccaacttagagatagaaagtctaaagttagatacagtgtggatacagtagtttcagaacttattagggaatacagtaataggtccgccattggcaacacaatcgaggctcttttccaaggtccacccaagttcaggccaattaggattagccttgaagagaaaccagctccggacgctattagcgatctccttgctagtgtagatagtgaagaagtgcgccaatactgcagggatcaaggctggatcattcctgaaactcccaccaacgtagagcggcaccttaatagagcagtgcttgtcatgcaatccatcaccacagtagtggcggttgtctcgttggtgtatgtcatctacaagctctttgcagggtttcagggtgcgtactctggtgctcctaagcaagtgcttaagaaacctgctcttcgcacagcaacagtacagggcccgagccttgattttgctctctccctgttgaggaggaacatcaggcaagtccaaacagaccaggggcatttcaccatgttgggtgttagggatcgtttagcagtcctcccgcgtcactcacaacccggtaaaactatttggattgagcataaactcgtgaacatccttgatgcagttgaattggtggatgagcaaggagtcaacctggaattaaccctcatcactcttgacactaacgaaaagtttagggatatcaccaaattcatcccagagaatattagcactgccagtgatgccactctagtgatcaacacggagcacatgccctcaatgtttgtcccggtgggtgacgttgtgcagtatggcttcttgaatctcagtggtaagcctacccatcgcaccatgatgtacaactttcctactaaagcagggcagtgtggaggagtggtgacatctgtcgggaaggttatcggtattcacattggtggcaatggtagacaaggtttttgcgcaggcctcaaaaggagttactttgctagtgaacaaggagagatccagtgggttaagcccaataaagaaactggaagacttaacatcaatggaccaacccgcaccaagttagaacccagtgtattccatgatgtcttcgagggaaataaggaaccagctgtcttgcacggtaaagatccccgactcgaggtagattttgagcaggccctgttctctaagtatgtgggaaatacactatatgagcctgacgagtacatcaaagaggcagcccttcattatgcaaatcaattaaagcaactagaaattaatacctctcaaatgagcatggaggaggcctgctacggtactgagaatcttgaggctattgatcttcatactagtgcaggttacccctatagtgccctgggaataaagaaaagagacatcttagaccctaccaccagggacgtgagtaaaatgaagttctacatggacaaatacggtcttgatctcccttactccacttatgtcaaggatgagctgcgctcaattgataaaattaggaaagggaagtcccgtctgatcgaggccagtagtttaaatgattcagtgtacctcagaatgactttcggccatttgtatgaggctttccacgcaaatcctgggacgataactggatcagccgtggggtgtaaccctgacacattctggagcaaactgccaatcttgctccctggttcactctttgcctttgactactcaggttatgatgctagccttagccctgtctggttcagagcattagaattggtccttagggagatagggtatagtgaaggcgcagtctcactcattgagggaatcaaccacacacaccatgtgtatcgcaatacgacctactgtgtgcttggtgggatgccctcaggctgttcgggaacatccattttcaactcaatgatcaacaacattattatcagggcactgctcataaaaacatttaagggcattgatttggacgaactcaacatggtcgcttatggagatgatgtgctcgccagctaccccttcccaattgattgcttggaattagcaaagactggcaaggagtatggtctaaccatgactcctgcagataagtctccttgctttaatgaagttaattggggtaatgcgaccttcctcaagaggggctttctacccgatgaacagtttccgtttttgatccaccctactatgccaatgagggagatccatgaatccattcgatggaccaaagacgcacgaaacactcaagatcatgtgcgatctttgtgcctcctagcatggcataatggtaagcaagaatatgagaaatttgtgagcacaattaggtctatcccagtaggaagagcgttggccatcccaaattatgaaaatcttagacgcaattggctcgagttattttagaggctacacgtacctcaaccccaccagaaatctggtcgtgaatatgactggtgggggtaaatttgttataaccagaatagcaaaaaaaaaaaaaaaaaaaaaaaaa

SEQ ID NO: 12 - DNA, 7448 bp, Enterovirus 71 C7/Osaka strain
ttaaaacagcctgtgggttgcacccactcacagggcccacgtggcgctagcactctgattccacggaacctttgtgcgcctgttttacgccccctccccaatttgcaacttagaagcaatacacaacactgatcaacagcaggcatggcacaccagctatgtcttgatcaagcacttctgtttccccggaccgagtatcaatagactgttcacgcggttgaaggagaaagcgtccgttatccggctaactacttcgagaaacctagtagcaccattgaagctgcagagtgtttcgctcggcacttcccccgtgtagatcaggtcgatgagtcactgcaatccccacgggcgaccgtggcagtggctgcgctggcggcctgcctatggggcaacccataggacgctctaatgtggacatggtgcgaagagtctattgagctagttagtagtcctccggcccctgaatgcggctaatcctaactgcggagcacatgccttcaatccagagggtggtgtgtcgtaatgggcaactctgcagcggaaccgactactttgggtgtccgtgtttccttttattcttacattggctgcttatggtgacaattgcagaattgttaccatatagctattggattggccatccggtgtgcaatagagctattatatacctatttgttggctttgtaccactaaccttaaaatctataaccaccctcgactttatattaaccctcaatacaatcaaacatgggctcacaggtgtctactcagcgatccggttcccacgagaactccaattcagctacagaaggctccaccattaattacactaccatcaactattacaaagactcctatgctgcgacagcgggcaaacaaagcctcaaacaagaccctgataagtttgctaaccctgtcaaggacattttcactgaaatggctgcgccactgaagtctccatccgctgaagcttgtggttacagtgatcgcgtggcacaactcaccattggaaactccaccattactacacaggaggcggcaaacatcatagtcggttatggtgagtggccctcatactgctctgatgacgatgctacagcggtggacaaaccaacgcgcccagatgtttcagtgaataggttttacacattggacactaaactgtgggaaaaatcatccaaggggtggtattggaagtttcctgatgtgttgactgagaccggagtctttggccagaacgcacagtttcactatttatatagatcagggttttgcattcatgtacaatgtaatgctagcaagttccatcaaggagcgctgttagtcgctatacttccagagtatgttatagggacagtagcaggcggcacaggaacagaggacagccaccctccttacaaacaaacacagcctggcgccgacggttttgagctgcagcacccgtacgtgctcgatgctgggattcctatatcacaattgacagtctgcccccatcaatggattaacctgcggaccaataactgtgccacaataatagtgccatatatgaatacactgcctttcgactctgccctgaaccattgcaattttgggctgttggtagtgcccattagcccattagactttgaccaaggggcaactccggttatccctattacaatcactctagctccaatgtgctctgagtttgcaggtctcagacaggcagtcacacaaggctttcccactgagccaaaaccaggaacgaatcaattcttgaccaccgatgacggcgtctcggcgcccattctaccaaatttccaccccactccatgtattcacatacccggtgaagtcagaaacctgcttgagttgtgtcaagtggagactattcttgaggttaacaacgtacccaccaatgctactagtctgatggaaaggctacgattcccagtgtccgcgcaagcggggaaaggtgaattgtgtgccgtgtttagggccgaccctggaagagacggcccatggcaatcaacaatgctgggccagttgtgtggatattacacccagtggtcagggtcactggaggtcacttttatgtttaccgggtcattcatggccacgggtaaaatgctcatagcttacacacctcctggcggcccattacctaaagatcgggccacagcaatgctgggcacacatgttatctgggattttgggctacaatcatctgtcacccttgtaataccatggatcagcaacacccactacagggcgcatgcccgggatggagtgttcgattactataccacaggactggtcagtatctggtatcaaacaaactatgtagttccaattggggcacccaacacagcttacataatagcactagcggcagcccagaagaattttaccatgaaactgtgcaaagacaccagccacatattacagacagcctctattcagggagatagggtggcagatgtgatcgagagctctataggagatagtgtgagtagggcacttacccaggccctgccagcacccacaggtcaaaacacacaggtgagtagtcatcgactagacactggcgaagttccagcgctccaagctgctgaaattggggcatcgtcaaatactagtgatgagagtatgattgaaacacgatgcgttcttaactcacacagtacagcggagaccaccttggacagcttcttcagtagggcaggtttggtaggagagatagatctccctcttgagggtaccactaatccaaatggttatgccaactgggacatagacataactggttacgcacaaatgcgcagaaaagtggagctgttcacctacatgcgctttgatgcggaattcacttttgttgcgtgcactcctactggtgaggttgttccacaattactccagtatatgtttgttccccctggtgctcccaaaccagagtctagagagtcacttgcttggcagacagccacaaacccctcagtttttgtcaagttgactgatcccccggcacaggtctcagttccgtttatgtcacccgcgagcgcttaccagtggttttacgacgggtaccccacgtttggagaacataaacaggagaaagaccttgagtatggagcgtgtcctaataatatgatgggcactttctcggtgcgaaccgtggggtcattaaagtccaagtaccctttggttgtcagaatatatatgagaatgaagcatgtcagggcgtggatacctcgcccgatgcgcaaccaaaactacttgttcaaagccaacccaaactatgccggtaactccattaaaccgaccggcactagtcgtactgccattactacccttggaaagttcggccagcaatctggggccatctacgtgggcaacttcagagtggttaatcgtcacctcgctactcacaatgactgggcgaatctcgtctgggaagacagctcccgcgacctattagtatcgtctaccaccgcccagggctgtgacacaattgcacgttgtgactgtcaaacaggagtgtactattgtaactccaagagaaagcactacccagtcagcttctctaaacccagcctcatatatgtggaagctagcgagtattaccctgctagataccaatcgcacctgatgcttgcagcgggccactctgagcccggtgactgcggaggcatcttaaggtgtcaacatggtgtagttggtatagtgtccacgggtggcaacgggctcgttggttttgctgatgtgagggatctcttgtggttagatgaagaggccatggagcaaggtgtgtccgactatattaaggggctcggtgacgcgtttggaacaggcttcaccgatgctgtatccagggaagttgaagcccttaggaaccacctcatagggtctgatggagcagttgagaaaatcctaaagaaccttatcaagctgatttcagcgttagtaattgtgatcaggagtgattatgatatggtcaccctcacagcaactttagccctgattggttgtcatggaagtccttgggcttggattaaagccaaaacagcatccattttaggtatccccatcgcccagaagcagagtgcttcttggctaaagaaatttaatgatatggcgagtgccgccaagggtttagaatggatatccaacaaaattagtaagttcattgactggctcagggagaagattgttccagcagctaaggagaaagcagaatttttaaccaatttgaagcaattaccactgttagagaaccagatcacgaatttagagcagtccgctgcctcacaagaggaccttgaagctatgtttgggaatgtgtcatacctcgcccatttctgtcgcaagttccaaccattatacgctacggaagctaagcgagtctatgttctagagaagagaatgaacaactacatgcagttcaagagcaaacaccgtattgaacctgtatgtctcatcattagaggctcaccgggcactggaaagtcccttgcgaccggtatcattgctcgggccatagcagacaagtatcactctagtgtgtactcacttccaccagatcctgaccattttgacgggtacaaacagcaagtggtcacagttatggatgatctgtgtcaaaatcctgacggcaaagacatgtcattattttgccagatggtgtccaccgtggattttatcccaccaatggcttctctcgaagaaaagggagtttctttcacatctaaatttgttatcgcatctaccaacgccagcaacattatagtgcctacagtgtctgactctgacgccattcgtcgcaggttttacatggattgcgacattgaggtgacagactcatacaaaacagacttgggtagactagacgctggacgggctgctaagttatgctctgaaaacaacaccgcaaacttcaaacgatgcagcccactagtgtgtgggaaagctattcaacttagggacaggaagtctaaggtcaggtacagcgtggacacagtggtttctgaacttattagagaacacaatagcagatccgctattggtaacacaattgaagcactattccaaggcccacccaagttcaggccaattagaatcagtcttgaagagaagccagccccagacgctattagcgatctcctcgctagtgtagacagcgaggaagtgcgccaatactgtagggagcaaggctggatcatccctgaaactcccaccaatgttgaacgacatcttaatagagcagtgctagtcatgcaatccatcgctactgtggtggcagtcgtctcactggtgtacgtcatttacaagctctttgcggggtttcaaggtgcgtattctggagctcccaagcaaatgctcaagaaacctgtcctccgcacggcaacagtacagggtccgagtcttgactttgctctatccttgctgagaaggaacatcaggcaagtccaaacagatcaagggcattttactatgttaggtgtcagggatcgcttggccgttctcccacggcactcacagcccgggaagactatttgggtggagcataaacttgtgaacatccttgacgcaatcgagctggtggatgagcagggcgttaatttggaactcacattggtgacactagatactaatgaaaaatttagagatatcaccaagttcattccagagaccattagcggcgctagtgatgcaactttagtgatcaacacagaacatatgccatcaatgtttgtcccagtgggggacgttgtgcagtacgggttcttgaaccttagtggaaagccaactcataggaccatgatgtacaatttccctacaaaagcaggacagtgtggaggtgtggtcacatcagtcggtaagattgtcggtatccacattggcggcaacgggcgccaggggttctgtgctggtctgaagaggagttacttcgcaagtgtgcagggtgagatccaatgggtgaagcctaacaaggaaactggtagactgaacatcaatggaccaactcgcactaagttggagcctagcgtatttcatgatgtgtttgaaggcaataaggaaccagcagttttaacaagtaaagaccctagattggaggtcgactttgagcaagccctgttttccaagtatgtgggcaatgttttacacgagcccgatgaatatgtgactcaagctgccctccactatgcgaatcaacttaaacaattggacataaacactagcaagatgagcatggaggaagcgtgctatggcactgaaaacctggaagcaatagacctctgcactagtgccggatatccatacagcgcccttggcattaagaaaagagacattctcgaccccacaaccagggatgtgtctaagatgaaattctatatggataaatacgggctagatctgccatactctacctatgtaaaggatgagcttaggtccctggataaaatcaagaaaggaaagtcacgcctgatagaggctagtagcttgaatgactctgtctacctcagaatgacttttgggcacctttacgaagtgtttcatgctaaccctggcactgtgactggctcagcagtgggttgcaacccggacgtgttttggagcaaactaccgattctgctgcctgggtcactctttgccttcgactactcaggatatgatgctagtctcagcccggtatggttcagggctctagaagttgtgttacgggagattgggtattcagaggaggccgtgtccctaatagaaggaatcaaccacacccaccatgtgtaccggaacaaaacatactgtgtacttggtggaatgccctcagggtgttctggtacttccatctttaatacaatgatcaacaacatcatcattagaacccttttgatcaaaacctttaagggaatagacctggatgagttgaacatggtggcctatggggacgatgtgctggctagttacccctttcctattgattgccttgagttggctaagactggcaaagagtatggtttgaccatgacacctgcagacaaatcaccctgtttcaatgaagtaacatgggaaaatgctaccttcctgaagagagggttcttgccagaccaccaatttccattcttaattcaccctacgatgcccatgagagagatccatgagtccattcgatggactaaagacgcgcgcaacacccaagatcacgtgcgctccctgtgtctgttggcatggcacaatggtaaggatgaatatgagaagtttgtgagtgcaattagatcagttccagttggaaaagcgttggccattcctaactttgagaatctgagaagaaattggctcgaattgttttaatattacagcttaaagctgaaccccactagaaatctggtcgtgttaatgactagtgggggtaaatttgttataaccagaatagcaaaaaaaaaaaaaaaaaaaaaaaaaaaaaaaaaaaa

SEQ ID NO: 13 - DNA, 7434 bp, Enterovirus 71 2716-Yamagata-03 strain
ttaaaacagcctgtgggttgcacccactcacaggacccacgtggtgctagcactctggttctacggaacccttgtgcgcctgttttacgccccctccccaatttgcaacttagaagcaattcacaacactgatcaatagcaggcatggcgcaccagctatgtcttgatcaagcacttctgtttccccggaccgagtatcaatagactgttcacgcggttgaaggagaaagcgtccgttatccggctaactacttcgagaaacccagtagcgccattgaaactgcagagtgtttcgctccacacttcccccgtgtagatcaggtcgatgagtcactgcaatccccacgggcgaccgtggcagtggctgcgctggcggcctgcctatggggcaacccataggacgctctaatgtggacatggtgcgaagagtctattgagctagttagtagtcctccggcccctgaatgcggctaatcctaactgcggagcacatgccttcaatccagagggtagtgtgtcgtaatgggcaactctgcagcggaaccgactactttgggtgtccgtgtttccttttattctcacattggctgcttatggtgacaattacagaattgttaccatatagctattggattggccatccggtgtgcaatagagctattatatacctatttgttggttttgtaccactaaccttaaaatctgcaaccactctcgactatatattaaccctcaatacaatcaaacatgggctcacaggtgtccactcaacgatccggctcccatgaaaactccaattcagctacagaaggctccaccattaattacaccactattaactattacaaagactcctatgctgcgacagcgggcaagcagagcctcaaacaagaccctgataagtttgctaaccctgtcaaggacattttcactgaaatggctgcgcctctaaagtctccatccgctgaagcttgtggctacagtgatcgcgtggcacaactcaccattggaaactccaccatcactacacaggaagcggcaaacatcatagtcggttatggtgaatggccctcatactgctctgatgacgacgctacagcggtggataagccaacgcgcccagatgtttccgtgaataggttttatacattggacactaaactatgggaaaagtcatccaaggggtggtattggaagtttcctgacgtattgactgagaccggagtctttggccaaaacgcacagtttcactatttatatagatcagggttttgcatccatgtgcaatgtaacgctagcaagttccaccaaggagcgctgttagtcgctatacttccagagtatgtcatagggacagtggcgggcggcacaggaacagaggacagtcaccctccttacaaacaaacacaaccaggtgccgacggttttgaattgcagcacccgtatgtgctcgatgctgggatccctatatcacaattgacagtatgcccccatcaatggattaacttacggactaataactgtgccacaataatagtgccatatatgaatacactgccttttgactccgccctgaaccattgcaattttgggctgttggtagtacccattagcccattagattttgaccaaggggcaactccggttatccctattacaatcactctagctccaatgtgctccgaatttgctggtctcaggcaggcagtcactcaaggctttcccactgagccaaaaccagggacgaatcaattcttgaccaccgatgatggcgtctcagcacccattctaccaaatttccatcccactccatgtattcacatacccggtgaagtcagaaacctgcttgagttgtgtcaagtggagactattcttgaggttaacaacgtacccaccaatgctactagtttgatggaaagactacgattcccggtgtccgcgcaagcggggaaaggtgaattgtgtgccgtgtttagggctgatcctggaagagacggtccatggcagtcaacgatgctgggccagttgtgtggatactacactcagtggtcagggtcactggaggtcactttcatgttcaccgggtctttcatggccacgggtaagatgctcatagcttatacaccccctggcggtcccttacccaaagatcgggctacagcaatgctgggcacacatgttatctgggactttgggctacaatcatctgtcacccttgtgataccatggatcagtaacactcactacagggcgcatgcccgggatggagtgttcgactactataccacaggactggtcagtatctggtatcaaacaaattatgtagtcccaattggggcacccaacacagcttacataatagcactggcggcggcccagaagaattttaccatgaaactgtgcaaagacactagtcacatactacagacagcctctattcagggagatagggtggcagatgtgatcgagagctctataggggacagcgtgggtagggcactcacccaggccctgccagcacccacaggtcaaaacacacaggtgagcagccatcgactagacactggtgaagttccagcgctccaagctgctgagatcggggcatcgtcaaatactagtgatgagagtatgattgagacacgatgcgtccttaactcacacagtacagcagagactaccctggacagtttctttagcagagcaggtttggtaggagagatagatctccctctagagggtactaccaatccaaatggttatgccaactgggatatagacataactggttatgcacaaatgcgcaggaaagtggagctgttcacctatatgcgctttgatgcggaattcactttcgttgcgtgcactcctactggtgaggttgttccacaactactccagtatatgtttgttccccctggtgctcctaaaccagagtctagagaatcacttgcttggcagacagccacaaacccttcagtttttgtcaaattaactgatcccccggcacaggtctcagttccgttcatgtcacccgcgagcgcttatcagtggttttacgacgggtaccccacgtttggagaacacaaacaggagaaagatcttgaatatggagcgtgtcctaacaacatgatgggcactttctcggtgcggaccgtggggtcttcgaaatccaagtaccctttggttgtcagaatatacatgagaatgaagcatgtcagggcatggatacctcgcccgatgcgcaaccaaaattacttgttcaaagccaatccaaattatgccggcaactccattaagccgaccggtactagtcgtaccgctattactacccttggaaagttcggccagcaatctggggccatctacgtgggcaacttcagagtggttaatcgtcacctcgctactcataatgactgggcaaacctcgtttgggaagacagctcccgcgacctattagtgtcgtctaccaccgcccagggctgtgatacaattgcacgttgtgactgtcaaacaggagtgtactattgtaactccaagagaaagcactatccagtcagcttttctaaacccagcctcatatatgtggaagctagcgagtattaccctgctaggtaccagtcgcacctgatgcttgcagcgggccactctgagcccggcgactgcggaggcatcttgaggtgtcaacatggtgtagttggtatagtgtccacgggtggcaacggactcgttggctttgctgatgtgagggacctcttgtggttagacgaagaagtcatggagcaaggtgtctccgactacattaaggggcttggtgacgcgtttgggacaggcttcaccgatgctgtgtccagggaagttgaagcccttaggaaccaccttataggatctgatggagcagttgagaaaatcctaaagaaccttattaagctgatttcagcgttagtaattgtgatcaggagcgattatgatatggtcaccctcacagctactttagccctgattggttgccatggaagtccttgggcttggatcaaagccaagacagcatccattttaggcatccccattgcccagaagcagagtgcttcttggctaaagaagttcaatgatatggcgagtgccgccaagggtttagagtggatatccaacaaaattagtaaattcattgactggctcagagagaagattgttccagcagctagagagaaagcagaattcttaaccaacttgaagcaattgccactgttagagaaccagatcacgaatttagaacagtccgctgcctcacaagaggaccttgaagccatgtttgggaatgtgtcatacctcgctcatttctgtcgcaagttccaaccattatacgccacagaagctaagcgggtctatgttctagagaagagaatgaacaactacatgcagttcaagagcaaacaccgtattgaacctgtatgtcttatcattagaggctcaccaggcactgggaagtcccttgcgaccggaatcattgctcgggccatagcagataagtatcactctagtgtgtactcacttccaccagaccctgaccattttgacgggtacaaacagcaagtggtcacagttatggatgatctgtgtcagaatcccgacggcaaggatatgtcgctattttgccagatggtgtccaccgtggattttatcccaccaatggcttctcttgaagaaaagggagtttcttttacatctaaatttgttattgcatccaccaacgccagcaacattatagtgcctacagtgtctgactctgacgccatccgacgcaggttttacatggattgcgacattgaggtgacggactcatataaaacagacttgggtagactagatgctggacgggctgctaagttatgctctgaaaacaacaccgcaaacttcaaacgatgcagccctctagtgtgtgggaaggctattcaacttagagacaggaagtccaaggtcaggtacagcgtggacacagtgatctctgaactaattagagaatacaatagcagatccgctattggtaacacaattgaagcactattccaaggcccgcctaagttcaggccaattagaatcagtcttgaggagaagccagccccagacgctattggcgatcttctcgctagtgtagacagcgaggaagtgcgccaatactgtagggagcaaggctggatcatccctgaaactcccaccaatgttgaacgacatcttaacagagcagtgctagttatgcaatccatcgctactgtggtggcagttgtctcactggtgtatgtcatttacaagctctttgcggggtttcaaggcgcgtattctggagctcccaagcaagtgctcaagaaacccgtcctccgcacggcaacagtgcagggtccaagtcttgactttgctctatccctgctgagaaggaacatcaggcaagtccaaacagatcaggggcattttaccatgttaggtgtcagggatcgcttagctgttctcccacggcacgcacagcccgggaagactatttgggtggagcacaagcttgtgaacgtcctcgacgcaatcgagctggtggatgaacagggcgttaatttggaactcacattggtgacactagacactaatgaaaaatttagagatatcaccaagttcattccagagaccattagcggcgctagtgatgcaactttagtgatcaatacagaacatatgccatcaatgtttgtcccagtgggggacgtcgtgcagtatgggttcttgaaccttagtgggaagccaacacataggaccatgatgtacaatttccctacaaaagcaggacaatgtggaggtgtggtcacatcagtcggtaagattgttggcattcacattggcggcaacgggcgccaagggttctgtgctggtttgaagaggagttacttcgcaagtgtgcagggtgagatccaatgggtgaagcctaacaaagaaactggtagactgaacatcaatggaccaactcgcactaagctggagcctagtgtgtttcatgatgtgtttgaaggcaataaggaaccagcagtcttaacaagtaaggaccctagattggaggtcgactttgagcaagccctgttttccaagtatgtgggcaatgttttacatgagcccgatgaatacgtgactcaagctgccctccactatgcgaatcaactcaaacagttggacataaacactagcaagatgagcatggaggaagcgtgctatggcactgagaacctggaagcaatagatctctgtactagtgccggatatccatacagcgcccttggcatcaagaaaagagacattctcgaccccgtaaccagggatgtgtctaagatgaaattctatatggataaatacgggctagatctgccatactccacctacgtgaaggatgagcttagatccctggataaaatcaagaaaggaaaatcacgcctgatagaggctagtagcttgaatgactctgtctacctcagaatgacctttgggcatctttacgaggtatttcatgctaaccctggcactgtgaccggttcggcagtgggttgcaacccagacgtgttttggagtaaactaccgatcctactgcctgggtcactctttgcctttgactactcaggatatgatgctagcctcagcccggtatggttcagggctctagaagttgtgttacgggaaattgggtatccagaggaggctgtgtccctaatagaaggaatcaaccacactcaccacgtgtaccggaacaaaacatattgtgtacttggtgggatgccttcagggtgttctggtacttccatctttaactcaatgatcaacaacatcatcattagaaccctcttaatcaaaacctttaagggaatagacctggatgagttgaacatggtggcctatggggacgatgtattggctagttatccctttcctatcgattgccttgagctggctaagactggcaaagagtatggtttgactatgacacctgcagacaaatcaccctgtttcaatgaagtgacatgggaaaatgctaccttccttaagagagggttcttgccagaccaccaatttccattcttaattcaccctacgatgcctatgagagagatccatgagtccattcgatggactaaagacgcacgcaatacccaagatcacgtgcgctctctgtgcctgttggcatggcacaatggtaaggatgaatatgaaaagtttgtgagtgcaattagatcagttccagttggaaaagcgttggccattcctaattttgagaatttgagaagaaattggctcgaattattttaacattacagcttaaagctgaaccccactagaaatctggtcgtgttaatgactagtgggggtaaatttgttataaccagaatagcaaaaaaaaaaaaaaaaaaaaaa

SEQ ID NO: 14 - DNA, 66 bp, Artificial Sequence
  EV71 Y90-3896 5'-primer
ctttcgtcttcaagaattgcggccgcgtaatacgactcactataggttaaaacagcctgtgggttg

SEQ ID NO: 15 - DNA, 59 bp, Artificial Sequence
  EV71 Y90-3896 3'-primer
gagaattgtcgaatatgtttaaactttttttttttttttttttttttttgctattctgg

SEQ ID NO: 16 - DNA, 52 bp, Artificial Sequence
  EV71 N772 5'-primer
ctaggcggccgcgtaatacgactcactataggttaaaacagcctgtgggttg

SEQ ID NO: 17 - DNA, 45 bp, Artificial Sequence
  EV71 N772 3'-primer
cacagtcgactttttttttttttttttttttttttgctattctgg

SEQ ID NO: 18 - DNA, 52 bp, Artificial Sequence; identical to SEQ ID NO: 16
  EV71 C7/Osaka 5'-primer

SEQ ID NO: 19 - DNA, 45 bp, Artificial Sequence
  EV71 C7/Osaka 3'-primer
cacactcgagtttttttttttttttttttttttttgctattctgg

SEQ ID NO: 20 - DNA, 66 bp, Artificial Sequence; identical to SEQ ID NO: 14
  EV71 2716-Yamagata 5'-primer

SEQ ID NO: 21 - DNA, 59 bp, Artificial Sequence; identical to SEQ ID NO: 15
  EV71 2716-Yamagata 3'-primer